European Patent Application EP 4 635 488 A1, published October 22, 2025. Title: Pharmaceutical compositions for preventing or treating bone diseases. Applicant: INDUSTRY FOUNDATION OF CHONNAM NATIONAL UNIVERSITY. The sequence listing filed with the application follows.

SEQUENCE LISTING (14 sequences)

SEQ ID NO: 1 - DNA, 21 bp, synthetic construct
  source 1..21: mol_type = other DNA
ggacgcagcgatgctaactaa

SEQ ID NO: 2 - DNA, 14 bp, synthetic construct
  source 1..14: mol_type = other DNA
cagagagaagggaa

SEQ ID NO: 3 - DNA, 19 bp, synthetic construct
  source 1..19: mol_type = other DNA
cagctgtcctggctcaaaa

SEQ ID NO: 4 - DNA, 20 bp, synthetic construct
  source 1..20: mol_type = other DNA
acatagcccacaccgttctc

SEQ ID NO: 5 - DNA, 20 bp, synthetic construct
  source 1..20: mol_type = other DNA
cgcacgatgcttcattcttc

SEQ ID NO: 6 - DNA, 17 bp, synthetic construct
  source 1..17: mol_type = other DNA
cagtgccagccgcaatc

SEQ ID NO: 7 - DNA, 20 bp, synthetic construct
  source 1..20: mol_type = other DNA
tgtgtccgtcgtggatctga

SEQ ID NO: 8 - DNA, 20 bp, synthetic construct
  source 1..20: mol_type = other DNA
gatgcctgcttcaccacctt

SEQ ID NO: 9 - DNA, 21 bp, synthetic construct
  source 1..21: mol_type = other DNA
ctggacagccagacactaaag

SEQ ID NO: 10 - DNA, 20 bp, synthetic construct
  source 1..20: mol_type = other DNA
ctcgcggcaagtcttcagag

SEQ ID NO: 11 - DNA, 18 bp, synthetic construct
  source 1..18: mol_type = other DNA
accacctttccgcaacca

SEQ ID NO: 12 - DNA, 23 bp, synthetic construct
  source 1..23: mol_type = other DNA
ggtactggcttctcttccgtttc

SEQ ID NO: 13 - DNA, 19 bp, synthetic construct
  source 1..19: mol_type = other DNA
actatggccacccgggaat

SEQ ID NO: 14 - DNA, 19 bp, synthetic construct
  source 1..19: mol_type = other DNA
ggcccaagggagtcatgtg